European Patent Application EP 4 230 217 A1, published August 23, 2023. Title: Pharmaceutical composition for preventing or treating lupus-associated diseases comprising GIP derivative or long acting conjugate thereof. Applicant: HANMI PHARM. CO., LTD. The sequence listing filed with the application follows.

SEQUENCE LISTING (46 sequences)

SEQ ID NO: 1 - protein, 40 aa, Artificial
  GIP derivative
  MISC_FEATURE (2)..(2): Xaa is aminoisobutyric acid (Aib)
YXEGTFISDYSIAMDAIAQQDFVNWLLAQKPSSGAPPPSC

SEQ ID NO: 2 - protein, 40 aa, Artificial
  GIP derivative
  MISC_FEATURE (2)..(2): Xaa is aminoisobutyric acid (Aib)
YXEGTFISDYSIAMDAIAQQDFVNWLLAGGPSSGAPPPSC

SEQ ID NO: 3 - protein, 40 aa, Artificial
  GIP derivative
  MISC_FEATURE (2)..(2): Xaa is aminoisobutyric acid (Aib)
  MISC_FEATURE (13)..(13): Xaa is aminoisobutyric acid (Aib)
YXEGTFISDYSIXMDAIAQQDFVNWLLAGGPSSGAPPPSC

SEQ ID NO: 4 - protein, 40 aa, Artificial
  GIP derivative
  MISC_FEATURE (2)..(2): Xaa is aminoisobutyric acid (Aib)
YXEGTFISDYSIYMDAIAQQDFVNWLLAGGPSSGAPPPSC

SEQ ID NO: 5 - protein, 40 aa, Artificial
  GIP derivative
  MISC_FEATURE (2)..(2): Xaa is aminoisobutyric acid (Aib)
YXEGTFISDYSIQMDAIAQQDFVNWLLAGGPSSGAPPPSC

SEQ ID NO: 6 - protein, 40 aa, Artificial
  GIP derivative
  MISC_FEATURE (2)..(2): Xaa is aminoisobutyric acid (Aib)
YXEGTFISDYSIYLDAIAQQDFVNWLLAGGPSSGAPPPSC

SEQ ID NO: 7 - protein, 40 aa, Artificial
  GIP derivative
  MISC_FEATURE (2)..(2): Xaa is aminoisobutyric acid (Aib)
YXEGTFISDYSIYLDAQAQQDFVNWLLAGGPSSGAPPPSC

SEQ ID NO: 8 - protein, 40 aa, Artificial
  GIP derivative
  MISC_FEATURE (2)..(2): Xaa is aminoisobutyric acid (Aib)
  MISC_FEATURE (20)..(20): Xaa is aminoisobutyric acid (Aib)
YXEGTFISDYSIYLDAQAAXDFVNWLLAGGPSSGAPPPSC

SEQ ID NO: 9 - protein, 40 aa, Artificial
  GIP derivative
  MISC_FEATURE (2)..(2): Xaa is aminoisobutyric acid (Aib)
YXEGTFISDYSIYLDAQAAKDFVNWLLAGGPSSGAPPPSC

SEQ ID NO: 10 - protein, 40 aa, Artificial
  GIP derivative
  MISC_FEATURE (2)..(2): Xaa is aminoisobutyric acid (Aib)
YXEGTFISDYSIYLDAQAAKEFIAWLLAGGPSSGAPPPSC

SEQ ID NO: 11 - protein, 43 aa, Artificial
  GIP derivative
  MISC_FEATURE (2)..(2): Xaa is aminoisobutyric acid (Aib)
YXEGTFISDYSIAMDAIAQQDFVNWLLAQKGKKNDWKHNITQC

SEQ ID NO: 12 - protein, 43 aa, Artificial
  GIP derivative
  MISC_FEATURE (2)..(2): Xaa is aminoisobutyric acid (Aib)
  MISC_FEATURE (20)..(20): Xaa is aminoisobutyric acid (Aib)
YXEGTFISDYSIYLDKQAAXEFVNWLLAQKGKKNDWKHNITQC

SEQ ID NO: 13 - protein, 31 aa, Artificial
  GIP derivative
  MISC_FEATURE (2)..(2): Xaa is aminoisobutyric acid (Aib)
  MISC_FEATURE (20)..(20): Xaa is aminoisobutyric acid (Aib)
YXEGTFISDYSIYLDKQAAXEFVNWLLAQKC

SEQ ID NO: 14 - protein, 31 aa, Artificial
  GIP derivative
  MISC_FEATURE (2)..(2): Xaa is aminoisobutyric acid (Aib)
  MISC_FEATURE (20)..(20): Xaa is aminoisobutyric acid (Aib)
YXEGTFISDYSIYLDAQAAXEFVNWLLAQKC

SEQ ID NO: 15 - protein, 40 aa, Artificial
  GIP derivative
  MISC_FEATURE (2)..(2): Xaa is aminoisobutyric acid (Aib)
YXEGTFISDYSIAMDKIAQQDFVNWLLAQKPSSGAPPPSC

SEQ ID NO: 16 - protein, 40 aa, Artificial
  GIP derivative
  MISC_FEATURE (2)..(2): Xaa is aminoisobutyric acid (Aib)
YXEGTFISDYSIAMDGIAQQDFVNWLLAQKPSSGAPPPSC

SEQ ID NO: 17 - protein, 40 aa, Artificial
  GIP derivative
  MISC_FEATURE (2)..(2): Xaa is aminoisobutyric acid (Aib)
YXEGTFISDYSIALEKQAQQDFVNWLLAGGPSSGAPPPSC

SEQ ID NO: 18 - protein, 40 aa, Artificial
  GIP derivative
  MISC_FEATURE (2)..(2): Xaa is aminoisobutyric acid (Aib)
YXEGTFISDYSIYLDKQAAQEFVNWLLAQKPSSGAPPPSC

SEQ ID NO: 19 - protein, 40 aa, Artificial
  GIP derivative
  MISC_FEATURE (2)..(2): Xaa is aminoisobutyric acid (Aib)
  MISC_FEATURE (20)..(20): Xaa is aminoisobutyric acid (Aib)
  MISC_FEATURE (28)..(28): Xaa is aminoisobutyric acid (Aib)
YXEGTFISDYSIYLDKQAAXEFVNWLLXGHPSSGAPPPSC

SEQ ID NO: 20 - protein, 40 aa, Artificial
  GIP derivative
  MISC_FEATURE (2)..(2): Xaa is aminoisobutyric acid (Aib)
  MISC_FEATURE (20)..(20): Xaa is aminoisobutyric acid (Aib)
  MISC_FEATURE (28)..(28): Xaa is aminoisobutyric acid (Aib)
YXEGTFISDYSIYLDKQAAXEFVNWLLXGGPSSGAPPPSC

SEQ ID NO: 21 - protein, 40 aa, Artificial
  GIP derivative
  MISC_FEATURE (2)..(2): Xaa is aminoisobutyric acid (Aib)
  MISC_FEATURE (13)..(13): Xaa is aminoisobutyric acid (Aib)
  MISC_FEATURE (20)..(20): Xaa is aminoisobutyric acid (Aib)
  MISC_FEATURE (28)..(28): Xaa is aminoisobutyric acid (Aib)
YXEGTFISDYSIXLDKQAAXEFVNWLLXGGPSSGAPPPSC

SEQ ID NO: 22 - protein, 40 aa, Artificial
  GIP derivative
  MISC_FEATURE (2)..(2): Xaa is aminoisobutyric acid (Aib)
  MISC_FEATURE (20)..(20): Xaa is aminoisobutyric acid (Aib)
YXEGTFISDYSIYLDKQAAXEFVNWLLAGHPSSGAPPPSC

SEQ ID NO: 23 - protein, 40 aa, Artificial
  GIP derivative
  MISC_FEATURE (2)..(2): Xaa is aminoisobutyric acid (Aib)
  MISC_FEATURE (28)..(28): Xaa is aminoisobutyric acid (Aib)
YXEGTFISDYSIYLDKQAQKEFVNWLLXGGPSSGAPPPSC

SEQ ID NO: 24 - protein, 40 aa, Artificial
  GIP derivative
  MISC_FEATURE (2)..(2): Xaa is aminoisobutyric acid (Aib)
  MISC_FEATURE (13)..(13): Xaa is aminoisobutyric acid (Aib)
  MISC_FEATURE (20)..(20): Xaa is aminoisobutyric acid (Aib)
  MISC_FEATURE (28)..(28): Xaa is aminoisobutyric acid (Aib)
YXEGTFISDYSIXLDKQAAXEFVNWLLXGHPSSGAPPPSC

SEQ ID NO: 25 - protein, 40 aa, Artificial
  GIP derivative
  MISC_FEATURE (2)..(2): Xaa is aminoisobutyric acid (Aib)
  MISC_FEATURE (20)..(20): Xaa is aminoisobutyric acid (Aib)
  MISC_FEATURE (28)..(28): Xaa is aminoisobutyric acid (Aib)
YXEGTFISDYSIYLDKQAAXEFVQWLIXGGPSSGAPPPSC

SEQ ID NO: 26 - protein, 39 aa, Artificial
  GIP derivative
  MISC_FEATURE (2)..(2): Xaa is aminoisobutyric acid (Aib)
  MISC_FEATURE (20)..(20): Xaa is aminoisobutyric acid (Aib)
YXEGTFISDYSIYLDKQAAXEFVQWLIAGHPSSGAPPPC

SEQ ID NO: 27 - protein, 12 aa, Homo sapiens
ESKYGPPCPSCP

SEQ ID NO: 28 - protein, 11 aa, Artificial
  Variant of hinge region
ESKYGPPPSCP

SEQ ID NO: 29 - protein, 11 aa, Artificial
  Variant of hinge region
ESKYGPPCPSP

SEQ ID NO: 30 - protein, 10 aa, Artificial
  Variant of hinge region
ESKYGPPCPS

SEQ ID NO: 31 - protein, 10 aa, Artificial
  Variant of hinge region
ESKYGPPCPP

SEQ ID NO: 32 - protein, 8 aa, Artificial
  Variant of hinge region
KYGPPCPS

SEQ ID NO: 33 - protein, 8 aa, Artificial
  Variant of hinge region
ESKYGPPC

SEQ ID NO: 34 - protein, 7 aa, Artificial
  Variant of hinge region
EKYGPPC

SEQ ID NO: 35 - protein, 6 aa, Artificial
  Variant of hinge region
ESPSCP

SEQ ID NO: 36 - protein, 5 aa, Artificial
  Variant of hinge region
EPSCP

SEQ ID NO: 37 - protein, 4 aa, Artificial
  Variant of hinge region
PSCP

SEQ ID NO: 38 - protein, 10 aa, Artificial
  Variant of hinge region
ESKYGPPSCP

SEQ ID NO: 39 - protein, 9 aa, Artificial
  Variant of hinge region
KYGPPPSCP

SEQ ID NO: 40 - protein, 9 aa, Artificial
  Variant of hinge region
ESKYGPSCP

SEQ ID NO: 41 - protein, 8 aa, Artificial
  Variant of hinge region
ESKYGPPC

SEQ ID NO: 42 - protein, 7 aa, Artificial
  Variant of hinge region
KYGPPCP

SEQ ID NO: 43 - protein, 7 aa, Artificial
  Variant of hinge region
ESKPSCP

SEQ ID NO: 44 - protein, 6 aa, Artificial
  Variant of hinge region
ESPSCP

SEQ ID NO: 45 - protein, 4 aa, Artificial
  Variant of hinge region
EPSC

SEQ ID NO: 46 - protein, 3 aa, Artificial
  Variant of hinge region
SCP